European Patent Application EP 4 656 245 A1, published December 3, 2025. Title: Histidine-Based Unnatural Amino Acid, its Production and Use. Applicant: Philipps-Universität Marburg. Application DE. The sequence listing filed with the application follows.

SEQUENCE LISTING (22 sequences)

SEQ ID NO: 1 - protein, 6 aa, synthetic construct
RRWWRF

SEQ ID NO: 2 - protein, 6 aa, synthetic construct
RRWWRB

SEQ ID NO: 3 - protein, 6 aa, synthetic construct
RRWWBF

SEQ ID NO: 4 - protein, 6 aa, synthetic construct
RRWBRF

SEQ ID NO: 5 - protein, 6 aa, synthetic construct
RRBWRF

SEQ ID NO: 6 - protein, 6 aa, synthetic construct
RBWWRF

SEQ ID NO: 7 - protein, 6 aa, synthetic construct
BRWWRF

SEQ ID NO: 8 - protein, 6 aa, synthetic construct
RRWWBB

SEQ ID NO: 9 - protein, 6 aa, synthetic construct
RRWBRB

SEQ ID NO: 10 - protein, 6 aa, synthetic construct
RRBWRB

SEQ ID NO: 11 - protein, 6 aa, synthetic construct
RBWWRB

SEQ ID NO: 12 - protein, 6 aa, synthetic construct
BRWWRB

SEQ ID NO: 13 - protein, 6 aa, synthetic construct
RRWBBF

SEQ ID NO: 14 - protein, 6 aa, synthetic construct
RRBWBF

SEQ ID NO: 15 - protein, 6 aa, synthetic construct
RBWWBF

SEQ ID NO: 16 - protein, 6 aa, synthetic construct
BRWWBF

SEQ ID NO: 17 - protein, 6 aa, synthetic construct
RRBBRF

SEQ ID NO: 18 - protein, 6 aa, synthetic construct
RBWBRF

SEQ ID NO: 19 - protein, 6 aa, synthetic construct
BRWBRF

SEQ ID NO: 20 - protein, 6 aa, synthetic construct
RBBWRF

SEQ ID NO: 21 - protein, 6 aa, synthetic construct
BRBWRF

SEQ ID NO: 22 - protein, 6 aa, synthetic construct
BBWWRF